European Patent Specification EP 2 919 826 B1, published June 11, 2025. Title: VASCULAR EMBOLIC SYSTEM. Applicant: 3-D MATRIX LTD. The sequence listing filed with the application follows.

SEQUENCE LISTING (58 sequences)

SEQ ID NO: 1 - protein, 4 aa, Artificial Sequence
  source: /note="Description of Artificial Sequence: Synthetic peptide"
RADA

SEQ ID NO: 2 - protein, 200 aa, Artificial Sequence
  source: /note="Description of Artificial Sequence: Synthetic polypeptide"
  VARIANT (9)..(200): /replace=" "
  misc_feature (1)..(200): /note="This sequence many encompass 2-50 'Arg-Ala-Asp-Ala' repeating units"
  misc_feature (1)..(200): /note="Variant residues given in the sequence have no preference with respect to those in the annotations for variant positions"
RADARADARADARADARADARADARADARADARADARADARADARADARADARADARADARADARADARADARADARADARADARADARADARADARADARADARADARADARADARADARADARADARADARADARADARADARADARADARADARADARADARADARADARADARADARADARADARADARADARADA

SEQ ID NO: 3 - protein, 4 aa, Artificial Sequence
  source: /note="Description of Artificial Sequence: Synthetic peptide"
IEIK

SEQ ID NO: 4 - protein, 200 aa, Artificial Sequence
  source: /note="Description of Artificial Sequence: Synthetic polypeptide"
  VARIANT (9)..(200): /replace=" "
  misc_feature (1)..(200): /note="This sequence many encompass 2-50 'Ile-Glu-Ile-Lys' repeating units"
  misc_feature (1)..(200): /note="Variant residues given in the sequence have no preference with respect to those in the annotations for variant positions"
IEIKIEIKIEIKIEIKIEIKIEIKIEIKIEIKIEIKIEIKIEIKIEIKIEIKIEIKIEIKIEIKIEIKIEIKIEIKIEIKIEIKIEIKIEIKIEIKIEIKIEIKIEIKIEIKIEIKIEIKIEIKIEIKIEIKIEIKIEIKIEIKIEIKIEIKIEIKIEIKIEIKIEIKIEIKIEIKIEIKIEIKIEIKIEIKIEIKIEIK

SEQ ID NO: 5 - protein, 4 aa, Artificial Sequence
  source: /note="Description of Artificial Sequence: Synthetic peptide"
KLDL

SEQ ID NO: 6 - protein, 200 aa, Artificial Sequence
  source: /note="Description of Artificial Sequence: Synthetic polypeptide"
  VARIANT (9)..(200): /replace=" "
  misc_feature (1)..(200): /note="This sequence many encompass 2-50 'Lys-Leu-Asp-Leu' repeating units"
  misc_feature (1)..(200): /note="Variant residues given in the sequence have no preference with respect to those in the annotations for variant positions"
KLDLKLDLKLDLKLDLKLDLKLDLKLDLKLDLKLDLKLDLKLDLKLDLKLDLKLDLKLDLKLDLKLDLKLDLKLDLKLDLKLDLKLDLKLDLKLDLKLDLKLDLKLDLKLDLKLDLKLDLKLDLKLDLKLDLKLDLKLDLKLDLKLDLKLDLKLDLKLDLKLDLKLDLKLDLKLDLKLDLKLDLKLDLKLDLKLDLKLDL

SEQ ID NO: 7 - protein, 16 aa, Artificial Sequence
  source: /note="Description of Artificial Sequence: Synthetic peptide"
RADARADARADARADA

SEQ ID NO: 8 - protein, 13 aa, Artificial Sequence
  source: /note="Description of Artificial Sequence: Synthetic peptide"
IEIKIEIKIEIKI

SEQ ID NO: 9 - protein, 17 aa, Artificial Sequence
  source: /note="Description of Artificial Sequence: Synthetic peptide"
IEIKIEIKIEIKIEIKI

SEQ ID NO: 10 - protein, 12 aa, Artificial Sequence
  source: /note="Description of Artificial Sequence: Synthetic peptide"
KLDLKLDLKLDL

SEQ ID NO: 11 - protein, 16 aa, Artificial Sequence
  source: /note="Description of Artificial Sequence: Synthetic peptide"
AEAEAKAKAEAEAKAK

SEQ ID NO: 12 - protein, 16 aa, Artificial Sequence
  source: /note="Description of Artificial Sequence: Synthetic peptide"
KAKAKAKAKAKAKAKA

SEQ ID NO: 13 - protein, 5 aa, Artificial Sequence
  source: /note="Description of Artificial Sequence: Synthetic peptide"
KAKAK

SEQ ID NO: 14 - protein, 16 aa, Artificial Sequence
  source: /note="Description of Artificial Sequence: Synthetic peptide"
AKAKAEAEAKAKAEAE

SEQ ID NO: 15 - protein, 16 aa, Artificial Sequence
  source: /note="Description of Artificial Sequence: Synthetic peptide"
AKAEAKAEAKAEAKAE

SEQ ID NO: 16 - protein, 8 aa, Artificial Sequence
  source: /note="Description of Artificial Sequence: Synthetic peptide"
AEAEAKAK

SEQ ID NO: 17 - protein, 12 aa, Artificial Sequence
  source: /note="Description of Artificial Sequence: Synthetic peptide"
AEAKAEAEAKAK

SEQ ID NO: 18 - protein, 16 aa, Artificial Sequence
  source: /note="Description of Artificial Sequence: Synthetic peptide"
KAEAKAEAKAEAKAEA

SEQ ID NO: 19 - protein, 16 aa, Artificial Sequence
  source: /note="Description of Artificial Sequence: Synthetic peptide"
AEAKAEAKAEAKAEAK

SEQ ID NO: 20 - protein, 8 aa, Artificial Sequence
  source: /note="Description of Artificial Sequence: Synthetic peptide"
ARARADAD

SEQ ID NO: 21 - protein, 16 aa, Artificial Sequence
  source: /note="Description of Artificial Sequence: Synthetic peptide"
ADADARARADADARAR

SEQ ID NO: 22 - protein, 16 aa, Artificial Sequence
  source: /note="Description of Artificial Sequence: Synthetic peptide"
ARADARADARADARAD

SEQ ID NO: 23 - protein, 16 aa, Artificial Sequence
  source: /note="Description of Artificial Sequence: Synthetic peptide"
DARADARADARADARA

SEQ ID NO: 24 - protein, 16 aa, Artificial Sequence
  source: /note="Description of Artificial Sequence: Synthetic peptide"
ADARADARADARADAR

SEQ ID NO: 25 - protein, 16 aa, Artificial Sequence
  source: /note="Description of Artificial Sequence: Synthetic peptide"
ARARADADARARADAD

SEQ ID NO: 26 - protein, 16 aa, Artificial Sequence
  source: /note="Description of Artificial Sequence: Synthetic peptide"
ARADAKAEARADAKAE

SEQ ID NO: 27 - protein, 16 aa, Artificial Sequence
  source: /note="Description of Artificial Sequence: Synthetic peptide"
AKAEARADAKAEARAD

SEQ ID NO: 28 - protein, 16 aa, Artificial Sequence
  source: /note="Description of Artificial Sequence: Synthetic peptide"
ARAKADAEARAKADAE

SEQ ID NO: 29 - protein, 16 aa, Artificial Sequence
  source: /note="Description of Artificial Sequence: Synthetic peptide"
AKARAEADAKARADAE

SEQ ID NO: 30 - protein, 16 aa, Artificial Sequence
  source: /note="Description of Artificial Sequence: Synthetic peptide"
AQAQAQAQAQAQAQAQ

SEQ ID NO: 31 - protein, 16 aa, Artificial Sequence
  source: /note="Description of Artificial Sequence: Synthetic peptide"
VQVQVQVQVQVQVQVQ

SEQ ID NO: 32 - protein, 16 aa, Artificial Sequence
  source: /note="Description of Artificial Sequence: Synthetic peptide"
YQYQYQYQYQYQYQYQ

SEQ ID NO: 33 - protein, 16 aa, Artificial Sequence
  source: /note="Description of Artificial Sequence: Synthetic peptide"
HQHQHQHQHQHQHQHQ

SEQ ID NO: 34 - protein, 16 aa, Artificial Sequence
  source: /note="Description of Artificial Sequence: Synthetic peptide"
ANANANANANANANAN

SEQ ID NO: 35 - protein, 16 aa, Artificial Sequence
  source: /note="Description of Artificial Sequence: Synthetic peptide"
VNVNVNVNVNVNVNVN

SEQ ID NO: 36 - protein, 16 aa, Artificial Sequence
  source: /note="Description of Artificial Sequence: Synthetic peptide"
YNYNYNYNYNYNYNYN

SEQ ID NO: 37 - protein, 16 aa, Artificial Sequence
  source: /note="Description of Artificial Sequence: Synthetic peptide"
HNHNHNHNHNHNHNHN

SEQ ID NO: 38 - protein, 16 aa, Artificial Sequence
  source: /note="Description of Artificial Sequence: Synthetic peptide"
ANAQANAQANAQANAQ

SEQ ID NO: 39 - protein, 16 aa, Artificial Sequence
  source: /note="Description of Artificial Sequence: Synthetic peptide"
AQANAQANAQANAQAN

SEQ ID NO: 40 - protein, 16 aa, Artificial Sequence
  source: /note="Description of Artificial Sequence: Synthetic peptide"
VNVQVNVQVNVQVNVQ

SEQ ID NO: 41 - protein, 16 aa, Artificial Sequence
  source: /note="Description of Artificial Sequence: Synthetic peptide"
VQVNVQVNVQVNVQVN

SEQ ID NO: 42 - protein, 16 aa, Artificial Sequence
  source: /note="Description of Artificial Sequence: Synthetic peptide"
YNYQYNYQYNYQYNYQ

SEQ ID NO: 43 - protein, 16 aa, Artificial Sequence
  source: /note="Description of Artificial Sequence: Synthetic peptide"
YQYNYQYNYQYNYQYN

SEQ ID NO: 44 - protein, 16 aa, Artificial Sequence
  source: /note="Description of Artificial Sequence: Synthetic peptide"
HNHQHNHQHNHQHNHQ

SEQ ID NO: 45 - protein, 16 aa, Artificial Sequence
  source: /note="Description of Artificial Sequence: Synthetic peptide"
HQHNHQHNHQHNHQHN

SEQ ID NO: 46 - protein, 18 aa, Artificial Sequence
  source: /note="Description of Artificial Sequence: Synthetic peptide"
AKAQADAKAQADAKAQAD

SEQ ID NO: 47 - protein, 18 aa, Artificial Sequence
  source: /note="Description of Artificial Sequence: Synthetic peptide"
VKVQVDVKVQVDVKVQVD

SEQ ID NO: 48 - protein, 18 aa, Artificial Sequence
  source: /note="Description of Artificial Sequence: Synthetic peptide"
YKYQYDYKYQYDYKYQYD

SEQ ID NO: 49 - protein, 18 aa, Artificial Sequence
  source: /note="Description of Artificial Sequence: Synthetic peptide"
HKHQHDHKHQHDHKHQHD

SEQ ID NO: 50 - protein, 28 aa, Unknown
  source: /note="Description of Unknown: Beta-amyloid peptide"
DAEFRHDSGYEVHHQKLVFFAEDVGSNK

SEQ ID NO: 51 - protein, 11 aa, Unknown
  source: /note="Description of Unknown: Beta-amyloid peptide"
GSNKGAIIGLM

SEQ ID NO: 52 - protein, 9 aa, Artificial Sequence
  source: /note="Description of Artificial Sequence: Synthetic peptide"
RPKQQFGLM

SEQ ID NO: 53 - protein, 11 aa, Artificial Sequence
  source: /note="Description of Artificial Sequence: Synthetic peptide"
  MOD_RES (1)..(1): D-Arg
  MOD_RES (7)..(7): D-Trp
  MOD_RES (9)..(9): D-Trp
RPKPQQWFWLL

SEQ ID NO: 54 - protein, 16 aa, Artificial Sequence
  source: /note="Description of Artificial Sequence: Synthetic peptide"
VRVRVDVDVRVRVDVD

SEQ ID NO: 55 - protein, 16 aa, Artificial Sequence
  source: /note="Description of Artificial Sequence: Synthetic peptide"
ADADAKAKADADAKAK

SEQ ID NO: 56 - protein, 16 aa, Artificial Sequence
  source: /note="Description of Artificial Sequence: Synthetic peptide"
EAEAEAEAEAEAEAEA

SEQ ID NO: 57 - protein, 16 aa, Artificial Sequence
  source: /note="Description of Artificial Sequence: Synthetic peptide"
ADADADADADADADAD

SEQ ID NO: 58 - protein, 16 aa, Artificial Sequence
  source: /note="Description of Artificial Sequence: Synthetic peptide"
  source: /note="N-term acetylated"
  source: /note="C-term amidated"
RADARADARADARADA